European Patent Specification EP 3 452 049 B1, published April 1, 2026. Title: GLP-1 RECEPTOR LIGAND MOIETY CONJUGATED OLIGONUCLEOTIDES AND USES THEREOF. Applicant: Ionis Pharmaceuticals, Inc. AstraZeneca AB. The sequence listing filed with the application follows.

SEQUENCE LISTING (79 sequences)

SEQ ID NO: 1 - protein, 31 aa, Artificial sequence
  Synthetic peptide
HAEGTFTSDVSSYLEGQAAKEFIAWLVKGRG

SEQ ID NO: 2 - protein, 30 aa, Artificial sequence
  Synthetic peptide
HAEGTFTSDVSSYLEGQAAKEFIAWLVKGR

SEQ ID NO: 3 - protein, 27 aa, Artificial sequence
  Synthetic peptide
EGTFTSDVSSYLEGQAAKEFIAWLVKG

SEQ ID NO: 4 - protein, 27 aa, Artificial sequence
  Synthetic peptide
EGTFTSDVSSYLEEQAAKEFIAWLVKG

SEQ ID NO: 5 - protein, 30 aa, Artificial Sequence
  Synthetic peptide
  MOD_RES (2)..(2): Aib
  MOD_RES (29)..(29): Aib
HXEGTFTSDVSSYLEGQAAREFIAFLVRXR

SEQ ID NO: 6 - protein, 31 aa, Artificial Sequence
  Synthetic peptide
  MOD_RES (2)..(2): Ala, Val, or Gly
  MOD_RES (16)..(16): Gly, Lys, or Glu
  MOD_RES (17)..(17): Gln or Lys
  MOD_RES (24)..(24): Ala or Glu
  MOD_RES (27)..(27): Val or Lys
  MOD_RES (28)..(28): Lys, Asn, or Arg
  MOD_RES (30)..(30): Arg or Gly
  MOD_RES (31)..(31): Gly, His, Pro, or not present
HXEGTFTSDVSSYLEXXAAKEFIXWLXXGXX

SEQ ID NO: 7 - protein, 31 aa, Artificial Sequence
  Synthetic peptide
HAEGTFTSDVSSYLEGQAAKEFIAWLVRGRG

SEQ ID NO: 8 - protein, 31 aa, Artificial Sequence
  Synthetic peptide
HAEGTFTSDVSSYLEGQAAKEFIEWLVKGRG

SEQ ID NO: 9 - protein, 31 aa, Artificial Sequence
  Synthetic peptide
HAEGTFTSDVSSYLEKQAAKEFIAWLVKGRG

SEQ ID NO: 10 - protein, 31 aa, Artificial Sequence
  Synthetic peptide
HGEGTFTSDVSSYLEEQAAKEFIAWLVKGGG

SEQ ID NO: 11 - protein, 31 aa, Artificial Sequence
  Synthetic peptide
HVEGTFTSDVSSYLEEQAAKEFIAWLVKGGG

SEQ ID NO: 12 - protein, 31 aa, Artificial Sequence
  Synthetic peptide
HGEGTFTSDVSSYLEEQAAKEFIAWLKNGGG

SEQ ID NO: 13 - protein, 31 aa, Artificial Sequence
  Synthetic peptide
HVEGTFTSDVSSYLEEQAAKEFIAWLKNGGG

SEQ ID NO: 14 - protein, 31 aa, Artificial Sequence
  Synthetic peptide
HGEGTFTSDVSSYLEEQAAKEFIAWLVKGGP

SEQ ID NO: 15 - protein, 31 aa, Artificial Sequence
  Synthetic peptide
HVEGTFTSDVSSYLEEQAAKEFIAWLVKGGP

SEQ ID NO: 16 - protein, 31 aa, Artificial Sequence
  Synthetic peptide
HGEGTFTSDVSSYLEEQAAKEFIAWLKNGGP

SEQ ID NO: 17 - protein, 31 aa, Artificial Sequence
  Synthetic peptide
HVEGTFTSDVSSYLEEQAAKEFIAWLKNGGP

SEQ ID NO: 18 - protein, 30 aa, Artificial Sequence
  Synthetic peptide
HGEGTFTSDVSSYLEEQAAKEFIAWLVKGG

SEQ ID NO: 19 - protein, 30 aa, Artificial Sequence
  Synthetic peptide
HVEGTFTSDVSSYLEEQAAKEFIAWLVKGG

SEQ ID NO: 20 - protein, 30 aa, Artificial Sequence
  Synthetic peptide
HVEGTFTSDVSSYLEEQAAKEFIAWLVNGG

SEQ ID NO: 21 - protein, 30 aa, Artificial Sequence
  Synthetic peptide
HGEGTFTSDVSSYLEEQAAKEFIAWLVNGG

SEQ ID NO: 22 - protein, 40 aa, Artificial sequence
  Synthetic peptide
  MOD_RES (2)..(2): Aib
HXEGTFTSDVSSYLEEQAAKEFIAWLVKGGPSSGAPPPSC

SEQ ID NO: 23 - protein, 40 aa, Artificial sequence
  Synthetic peptide
  MOD_RES (2)..(2): Aib
  misc_feature (40)..(40): Xaa is Penicillamine (Pen)
HXEGTFTSDVSSYLEEQAAKEFIAWLVKGGPSSGAPPPSX

SEQ ID NO: 24 - protein, 31 aa, Artificial sequence
  Synthetic peptide
HAEGTFTSDVSSYLEGQAAKEFIAWLVKGRC

SEQ ID NO: 25 - protein, 39 aa, Artificial sequence
  Synthetic peptide
HGEGTFTSDLSKQMEEEAVRLFIEWLKNGGPSSGAPPPS

SEQ ID NO: 26 - protein, 40 aa, Artificial sequence
  Synthetic peptide
AGEGTFTSDVSSYLEGQAAKEAIAWLVKGGPSSGAPPPSC

SEQ ID NO: 27 - protein, 40 aa, Artificial sequence
  Synthetic peptide
  misc_feature (40)..(40): Xaa is Penicillamine (Pen)
AGEGTFTSDVSSYLEGQAAKEAIAWLVKGGPSSGAPPPSX

SEQ ID NO: 28 - protein, 27 aa, Artificial sequence
  Synthetic peptide
  MOD_RES (2)..(2): Aib
HXEGTFTSDVSSYLEEQAAKEFIAWLV

SEQ ID NO: 29 - protein, 28 aa, Artificial sequence
  Synthetic peptide
  MOD_RES (2)..(2): Aib
HXEGTFTSDVSSYLEEQAAKEFIAWLVK

SEQ ID NO: 30 - protein, 29 aa, Artificial sequence
  Synthetic peptide
  MOD_RES (2)..(2): Aib
HXEGTFTSDVSSYLEEQAAKEFIAWLVKG

SEQ ID NO: 31 - protein, 30 aa, Artificial sequence
  Synthetic peptide
  MOD_RES (2)..(2): Aib
HXEGTFTSDVSSYLEEQAAKEFIAWLVKGG

SEQ ID NO: 32 - protein, 31 aa, Artificial sequence
  Synthetic peptide
  MOD_RES (2)..(2): Aib
HXEGTFTSDVSSYLEEQAAKEFIAWLVKGGP

SEQ ID NO: 33 - protein, 32 aa, Artificial sequence
  Synthetic peptide
  MOD_RES (2)..(2): Aib
HXEGTFTSDVSSYLEEQAAKEFIAWLVKGGPS

SEQ ID NO: 34 - protein, 33 aa, Artificial sequence
  Synthetic peptide
  MOD_RES (2)..(2): Aib
HXEGTFTSDVSSYLEEQAAKEFIAWLVKGGPSS

SEQ ID NO: 35 - protein, 34 aa, Artificial sequence
  Synthetic peptide
  MOD_RES (2)..(2): Aib
HXEGTFTSDVSSYLEEQAAKEFIAWLVKGGPSSG

SEQ ID NO: 36 - protein, 35 aa, Artificial sequence
  Synthetic peptide
  MOD_RES (2)..(2): Aib
HXEGTFTSDVSSYLEEQAAKEFIAWLVKGGPSSGA

SEQ ID NO: 37 - protein, 36 aa, Artificial sequence
  Synthetic peptide
  MOD_RES (2)..(2): Aib
HXEGTFTSDVSSYLEEQAAKEFIAWLVKGGPSSGAP

SEQ ID NO: 38 - protein, 40 aa, Artificial sequence
  Synthetic peptide
  MOD_RES (40)..(40): Xaa is 4-azidonorleucine
HGEGTFTSDLSKQMEEEAVRLFIEWLKNGGPSSGAPPPSX

SEQ ID NO: 39 - protein, 32 aa, Artificial sequence
  Synthetic peptide
  MOD_RES (2)..(2): Aib
  MOD_RES (32)..(32): Xaa is 4-azidonorleucine
HXEGTFTSDVSSYLEGQAAKEFIAWLVRGRGX

SEQ ID NO: 40 - protein, 32 aa, Artificial sequence
  Synthetic peptide
  MOD_RES (2)..(2): Aib
  MOD_RES (21)..(21): Xaa is Lysine (5 azido pentanoic acid amide)
HXEGTFTSDVSSYLEGQAANXEFIAWLVRGRG

SEQ ID NO: 41 - protein, 31 aa, Artificial sequence
  Synthetic peptide
  MOD_RES (2)..(2): Aib
  MOD_RES (29)..(29): Aib
  MOD_RES (31)..(31): Xaa is 4-azidonorleucine
HXEGTFTSDVSSYLEGQAAKEFIAWLVKXRX

SEQ ID NO: 42 - protein, 31 aa, Artificial sequence
  Synthetic peptide
  MOD_RES (31)..(31): Xaa is 4-azidonorleucine
HSEGTFTSDVSSYLEGQAAKEFIAWLVKGRX

SEQ ID NO: 43 - protein, 38 aa, Artificial sequence
  Synthetic peptide
  MOD_RES (2)..(2): Aib
  MOD_RES (38)..(38): Xaa is 4-azidonorleucine
HXEGTFTSDVSSYLEEQAAKEFIAWLVKGGPSSGAPPX

SEQ ID NO: 44 - protein, 34 aa, Artificial sequence
  Synthetic peptide
  MOD_RES (2)..(2): Aib
  MOD_RES (44)..(44): Xaa is 4-azidonorleucine
HXEGTFTSDVSSYLEEQAAKEFIAWLVKGGPSSX

SEQ ID NO: 45 - protein, 29 aa, Artificial sequence
  Synthetic peptide
  MOD_RES (2)..(2): Aib
  MOD_RES (29)..(29): Xaa is 4-azidonorleucine
HXEGTFTSDVSSYLEEQAAKEFIAWLVKX

SEQ ID NO: 46 - protein, 28 aa, Artificial sequence
  Synthetic peptide
  MOD_RES (2)..(2): Aib
  MOD_RES (28)..(28): Xaa is 4-azidonorleucine
HXEGTFTSDVSSYLEEQAAKEFIAWLVX

SEQ ID NO: 47 - protein, 28 aa, Artificial sequence
  Synthetic peptide
  MOD_RES (2)..(2): Aib
HXEGTFTSDVSSYLEEQAAKEFIAWLVC

SEQ ID NO: 48 - protein, 27 aa, Artificial sequence
  Synthetic peptide
  MOD_RES (2)..(2): Aib
  MOD_RES (27)..(27): Xaa is 4-azidonorleucine
HXEGTFTSDVSSYLEEQAAKEFIAWLX

SEQ ID NO: 49 - protein, 26 aa, Artificial sequence
  Synthetic peptide
  MOD_RES (2)..(2): Aib
  MOD_RES (26)..(26): Xaa is 4-azidonorleucine
HXEGTFTSDVSSYLEEQAAKEFIAWX

SEQ ID NO: 50 - protein, 20 aa, Artificial sequence
  Synthetic peptide
  MOD_RES (2)..(2): Aib
  MOD_RES (20)..(20): Xaa is 4-azidonorleucine
HXEGTFTSDVSSYLEEQAAX

SEQ ID NO: 51 - protein, 30 aa, Artificial sequence
  Synthetic peptide
  MOD_RES (30)..(30): Xaa is 4-azidonorleucine
HGEGTFTSDLSKQMEEEAVRLFIEWLKNGX

SEQ ID NO: 52 - protein, 29 aa, Artificial sequence
  Synthetic peptide
  MOD_RES (29)..(29): Xaa is 4-azidonorleucine
HGEGTFTSDLSKQMEEEAVRLFIEWLKNX

SEQ ID NO: 53 - protein, 28 aa, Artificial sequence
  Synthetic peptide
  MOD_RES (28)..(28): Xaa is 4-azidonorleucine
HGEGTFTSDLSKQMEEEAVRLFIEWLKX

SEQ ID NO: 54 - protein, 27 aa, Artificial sequence
  Synthetic peptide
  MOD_RES (27)..(27): Xaa is 4-azidonorleucine
HGEGTFTSDLSKQMEEEAVRLFIEWLX

SEQ ID NO: 55 - protein, 26 aa, Artificial sequence
  Synthetic peptide
  MOD_RES (26)..(26): Xaa is 4-azidonorleucine
HGEGTFTSDLSKQMEEEAVRLFIEWX

SEQ ID NO: 56 - protein, 40 aa, Artificial sequence; identical to SEQ ID NO: 23
  Synthetic peptide
  MOD_RES (2)..(2): Aib
  MOD_RES (40)..(40): Xaa is 4-azidonorleucine

SEQ ID NO: 57 - protein, 40 aa, Artificial sequence
  Synthetic peptide
HGEGTFTSDLSKQMEEEAVRLFIEWLKNGGPSSGAPPPSC

SEQ ID NO: 58 - DNA, 19 bp, Artificial sequence
  Synthetic oligonucleotide
tcagcattctaatagcagc

SEQ ID NO: 59 - DNA, 19 bp, Artificial sequence
  Synthetic oligonucleotide
tcatcttcttaaaataccc

SEQ ID NO: 60 - DNA, 19 bp, Artificial sequence
  Synthetic oligonucleotide
tcaggccaatacgccgtca

SEQ ID NO: 61 - DNA, 23 bp, Artificial sequence
  Synthetic oligonucleotide
tcagccaaggtctgaaggtcacc

SEQ ID NO: 62 - DNA, 16 bp, Artificial sequence
  Synthetic oligonucleotide
gctgctattagaatgc

SEQ ID NO: 63 - DNA, 16 bp, Artificial sequence
  Synthetic oligonucleotide
gcattctaatagcagc

SEQ ID NO: 64 - DNA, 16 bp, Artificial sequence
  Synthetic oligonucleotide
tcttcttaaaataccc

SEQ ID NO: 65 - DNA, 16 bp, Artificial sequence
  Synthetic oligonucleotide
gcattctaatagcagc

SEQ ID NO: 66 - DNA, 24 bp, Artificial sequence
  Primer
ccattctatcatcaacgggtacaa

SEQ ID NO: 67 - DNA, 22 bp, Artificial sequence
  Primer
agcaagtgggaaggtgtaatcc

SEQ ID NO: 68 - DNA, 20 bp, Artificial sequence
  Primer
cagtcacatacggccaatcc

SEQ ID NO: 69 - DNA, 24 bp, Artificial sequence
  Primer
cgtaacttgatttgctgtcctgaa

SEQ ID NO: 70 - DNA, 25 bp, Artificial sequence
  Probe
tgagccctttgccccagatgcctat

SEQ ID NO: 71 - DNA, 24 bp, Artificial sequence
  Primer
gaggaatcagatgaggatatggga

SEQ ID NO: 72 - DNA, 20 bp, Artificial sequence
  Primer
aagcaggctgacttggttgc

SEQ ID NO: 73 - DNA, 26 bp, Artificial sequence
  Probe
tcggtctcttcgactaatcccgccaa

SEQ ID NO: 74 - DNA, 20 bp, Artificial sequence
  Primer
aggcgttgtgcgtagaggat

SEQ ID NO: 75 - DNA, 29 bp, Artificial sequence
  Primer
aaaggttaccataagtaagttccagaaaa

SEQ ID NO: 76 - DNA, 28 bp, Artificial sequence
  Probe
agtggttggtaaaaatccgtgaggtcgg

SEQ ID NO: 77 - DNA, 21 bp, Artificial sequence
  siRNA
ttatctataatgatcaggtaa

SEQ ID NO: 78 - DNA, 19 bp, Artificial sequence
  siRNA
acctgatcattatagataa

SEQ ID NO: 79 - protein, 32 aa, Artificial sequence
  Synthetic peptide
DLSKQMEEEAVRLFIEWLKNGGPSSGAPPPSC